European Patent Specification EP 3 774 859 B1, published March 13, 2024. Title: HUMAN NEUREGULIN-1 (NRG-1) RECOMBINANT FUSION PROTEIN COMPOSITIONS AND METHODS OF USE THEREOF. Applicant: Salubris Biotherapeutics, Inc. Genekey Biotech (Chengdu) Co., Ltd. The sequence listing filed with the application follows.

SEQUENCE LISTING (18 sequences)

SEQ ID NO: 1 - protein, 331 aa, Homo sapiens
MRANDALQVLGLLFSLARGSEVGNSQAVCPGTLNGLSVTGDAENQYQTLYKLYERCEVVMGNLEIVLTGHNADLSFLQWIREVTGYVLVAMNEFSTLPLPNLRVVRGTQVYDGKFAIFVMLNYNTNSSHALRQLRLTQLTEILSGGVYIEKNDKLCHMDTIDWRDIVRDRDAEIVVKDNGRSCPPCHEVCKGRCWGPGSEDCQTLTKTICAPQCNGHCFGPNPNQCCHDECAGGCSGPQDTDCFACRHFNDSGACVPRCPQPLVYNKLTFQLEPNPHTKYQYGGVCVASCPHNFVVDQTSCVRACPPDKMEVDKNGLKMCEPCGGLCPKAF

SEQ ID NO: 2 - protein, 447 aa, Homo sapiens
QVQLQQWGAGLLKPSETLSLTCAVYGGSFSGYYWSWIRQPPGKGLEWIGEINHSGSTNYNPSLKSRVTISVETSKNQFSLKLSSVTAADTAVYYCARDKWTWYFDLWGRGTLVTVSSASTKGPSVFPLAPSSKSTSGGTAALGCLVKDYFPEPVTVSWNSGALTSGVHTFPAVLQSSGLYSLSSVVTVPSSSLGTQTYICNVNHKPSNTKVDKRVEPKSCDKTHTCPPCPAPEFLGGPAVFLFPPKPKDTLMISRTPEVTCVVVDVSHEDPEVKFNWYVDGVEVHNAKTKPREEQYNSTYRVVSVLTVLHQDWLNGKEYKCKVSNKALPAPIEKTISKAKGQPREPQVYTLPPSREEMTKNQVSLTCLVKGFYPSDIAVEWESNGQPENNYKTTPPVLDSDGSFFLYSKLTVDKSRWQQGNVFSCSVMHEALHAHYTQKSLSLSPGK

SEQ ID NO: 3 - protein, 220 aa, Homo sapiens
DIEMTQSPDSLAVSLGERATINCRSSQSVLYSSSNRNYLAWYQQNPGQPPKLLIYWASTRESGVPDRFSGSGSGTDFTLTISSLQAEDVAVYYCQQYYSTPRTFGQGTKVEIKRTVAAPSVFIFPPSDEQLKSGTASVVCLLNNFYPREAKVQWKVDNALQSGNSQESVTEQDSKDSTYSLSSTLTLSKADYEKHKVYACEVTHQGLSSPVTKSFNRGEC

SEQ ID NO: 4 - protein, 61 aa, Homo sapiens
SHLVKCAEKEKTFCVNGGECFMVKDLSNPSRYLCKCPNEFTGDRCQNYVMASFYKAEELYQ

SEQ ID NO: 5 - protein, 10 aa, Artificial
  Glycine-Serine linker
GGGGSGGGGS

SEQ ID NO: 6 - DNA, 1614 bp, Homo sapiens
atggagtttgggctgagctgggttttccttgttgctataataaaaggtgtccagtgtcaggtgcagctgcagcagtggggagctggactgctgaagccaagcgagaccctgtctctgacatgcgccgtgtacggaggatccttcagcggatactattggtcttggatcaggcagccacctggcaagggactggagtggatcggcgagatcaaccactctggctccaccaactacaatccctctctgaagtcccgggtgaccatctccgtggagacaagcaagaatcagttttccctgaagctgtccagcgtgaccgccgctgacacagccgtgtactattgcgctagggacaagtggacctggtatttcgatctgtggggaaggggcaccctggtgacagtgtcttccgcctctacaaagggcccctccgtgtttcctctggctccaagctctaagagcacctctggaggaacagccgctctgggatgtctggtgaaggattacttccctgagccagtgaccgtgagctggaactctggcgccctgacctccggagtgcatacatttcccgctgtgctgcagtccagcggcctgtatagcctgtcttccgtggtgaccgtgcctagctcttccctgggcacccagacatacatctgcaacgtgaatcacaagccctccaatacaaaggtggacaagagagtggagcctaagagctgtgataagacccatacatgcccaccatgtccagctcctgagctgctgggaggaccttccgtgttcctgtttcctccaaagccaaaggacaccctgatgatctctcgcacccctgaggtgacatgcgtggtggtggacgtgtcccacgaggatccagaggtgaagttcaactggtacgtggatggcgtggaggtgcataatgctaagaccaagcctagggaggagcagtacaacagcacctatcgggtggtgtctgtgctgacagtgctgcaccaggactggctgaacggcaaggagtacaagtgcaaggtgagcaataaggccctgccagctcccatcgagaagaccatctctaaggccaagggccagcccagagagcctcaggtgtatacactgccccctagccgcgaggagatgaccaagaaccaggtgtctctgacatgtctggtgaagggcttctacccatctgacatcgctgtggagtgggagtccaatggccagcccgagaacaattataagaccacaccacccgtgctggactccgatggcagcttctttctgtactccaagctgaccgtggataagagcaggtggcagcagggcaacgtgttttcctgcagcgtgatgcacgaggccctgcacaatcattatacacagaaatctctgtccctgagcccaggcaagggaggaggaggaagcggaggaggaggcagctctcatctggtgaagtgtgctgagaaggagaagaccttctgcgtgaacggcggcgagtgttttatggtgaaggacctgtctaatccatccagatacctgtgcaagtgtcccaacgagttcacaggcgatcgctgccagaattacgtgatggcctctttttataaggctgaggagctgtaccagtaa

SEQ ID NO: 7 - DNA, 1614 bp, Homo sapiens
atggagtttgggctgagctgggttttccttgttgctataataaaaggtgtccagtgtcaggtgcagctgcagcagtggggagctggactgctgaagccaagcgagaccctgtctctgacatgcgccgtgtacggaggatccttcagcggatactattggtcttggatcaggcagccacctggcaagggactggagtggatcggcgagatcaaccactctggctccaccaactacaatccctctctgaagtcccgggtgaccatctccgtggagacaagcaagaatcagttttccctgaagctgtccagcgtgaccgccgctgacacagccgtgtactattgcgctagggacaagtggacctggtatttcgatctgtggggaaggggcaccctggtgacagtgtcttccgcctctacaaagggcccctccgtgtttcctctggctccaagctctaagagcacctctggaggaacagccgctctgggatgtctggtgaaggattacttccctgagccagtgaccgtgagctggaactctggcgccctgacctctggagtgcatacatttcccgctgtgctgcagtccagcggcctgtatagcctgtcttccgtggtgaccgtgcctagctcttccctgggcacccagacatacatctgcaacgtgaatcacaagccctccaatacaaaggtggacaagagagtggagcctaagagctgtgataagacccatacatgcccaccatgtccagctcctgagttcctgggaggacctgccgtgttcctgtttcctccaaagccaaaggacaccctgatgatctctcgcacccctgaggtgacatgcgtggtggtggacgtgtcccacgaggatccagaggtgaagttcaactggtacgtggatggcgtggaggtgcataatgctaagaccaagcctagggaggagcagtacaacagcacctatcgggtggtgtctgtgctgacagtgctgcaccaggactggctgaacggcaaggagtacaagtgcaaggtgagcaataaggccctgccagctcccatcgagaagaccatctctaaggccaagggccagcccagagagcctcaggtgtatacactgccccctagccgcgaggagatgaccaagaaccaggtgtctctgacctgtctggtgaagggcttctacccatctgacatcgctgtggagtgggagtccaatggccagcccgagaacaattataagaccacaccacccgtgctggactccgatggcagcttctttctgtactccaagctgaccgtggataagagcaggtggcagcagggcaacgtgttttcctgcagcgtgatgcacgaggccctgcacgctcattatacacagaaatctctgtccctgagcccaggcaagggaggaggaggaagcggaggaggaggcagctctcatctggtgaagtgtgctgagaaggagaagaccttctgcgtgaacggcggcgagtgttttatggtgaaggacctgtctaatccatccagatacctgtgcaagtgtcccaacgagttcacaggcgatcgctgccagaattacgtgatggcctctttttataaggctgaggagctgtaccagtaa

SEQ ID NO: 8 - DNA, 723 bp, Homo sapiens
atggtgttgcagacccaggtcttcatttctctgttgctctggatctctggtgcctacggggacatcgagatgacccagtctccagattccctggccgtgagcctgggagagagggctacaatcaactgccggtccagccagtctgtgctgtactcttccagcaacaggaattacctggcctggtatcagcagaatcccggccagccccctaagctgctgatctattgggctagcaccagagagtctggagtgcctgaccgcttctctggatccggaagcggcacagacttcaccctgacaatctcttccctgcaggccgaggacgtggccgtgtactattgccagcagtattactctacccctaggacattcggccagggcaccaaggtggagatcaagcggacagtggccgctccatccgtgttcatctttccaccctccgacgagcagctgaagtccggaaccgctagcgtggtgtgcctgctgaacaacttctacccaagagaggccaaggtgcagtggaaggtggataacgctctgcagagcggcaattctcaggagtccgtgaccgagcaggacagcaaggattctacatattccctgagctctaccctgacactgtccaaggccgattacgagaagcacaaggtgtatgcttgcgaggtgacccatcagggcctgtccagccccgtgacaaagagcttcaaccgcggcgagtgttaa

SEQ ID NO: 9 - protein, 537 aa, Homo sapiens
MEFGLSWVFLVAIIKGVQCQVQLQQWGAGLLKPSETLSLTCAVYGGSFSGYYWSWIRQPPGKGLEWIGEINHSGSTNYNPSLKSRVTISVETSKNQFSLKLSSVTAADTAVYYCARDKWTWYFDLWGRGTLVTVSSASTKGPSVFPLAPSSKSTSGGTAALGCLVKDYFPEPVTVSWNSGALTSGVHTFPAVLQSSGLYSLSSVVTVPSSSLGTQTYICNVNHKPSNTKVDKRVEPKSCDKTHTCPPCPAPELLGGPSVFLFPPKPKDTLMISRTPEVTCVVVDVSHEDPEVKFNWYVDGVEVHNAKTKPREEQYNSTYRVVSVLTVLHQDWLNGKEYKCKVSNKALPAPIEKTISKAKGQPREPQVYTLPPSREEMTKNQVSLTCLVKGFYPSDIAVEWESNGQPENNYKTTPPVLDSDGSFFLYSKLTVDKSRWQQGNVFSCSVMHEALHNHYTQKSLSLSPGKGGGGSGGGGSSHLVKCAEKEKTFCVNGGECFMVKDLSNPSRYLCKCPNEFTGDRCQNYVMASFYKAEELYQ

SEQ ID NO: 10 - protein, 537 aa, Homo sapiens
MEFGLSWVFLVAIIKGVQCQVQLQQWGAGLLKPSETLSLTCAVYGGSFSGYYWSWIRQPPGKGLEWIGEINHSGSTNYNPSLKSRVTISVETSKNQFSLKLSSVTAADTAVYYCARDKWTWYFDLWGRGTLVTVSSASTKGPSVFPLAPSSKSTSGGTAALGCLVKDYFPEPVTVSWNSGALTSGVHTFPAVLQSSGLYSLSSVVTVPSSSLGTQTYICNVNHKPSNTKVDKRVEPKSCDKTHTCPPCPAPEFLGGPAVFLFPPKPKDTLMISRTPEVTCVVVDVSHEDPEVKFNWYVDGVEVHNAKTKPREEQYNSTYRVVSVLTVLHQDWLNGKEYKCKVSNKALPAPIEKTISKAKGQPREPQVYTLPPSREEMTKNQVSLTCLVKGFYPSDIAVEWESNGQPENNYKTTPPVLDSDGSFFLYSKLTVDKSRWQQGNVFSCSVMHEALHAHYTQKSLSLSPGKGGGGSGGGGSSHLVKCAEKEKTFCVNGGECFMVKDLSNPSRYLCKCPNEFTGDRCQNYVMASFYKAEELYQ

SEQ ID NO: 11 - protein, 19 aa, Homo sapiens
MEFGLSWVFLVAIIKGVQC

SEQ ID NO: 12 - protein, 240 aa, Homo sapiens
MVLQTQVFISLLLWISGAYGDIEMTQSPDSLAVSLGERATINCRSSQSVLYSSSNRNYLAWYQQNPGQPPKLLIYWASTRESGVPDRFSGSGSGTDFTLTISSLQAEDVAVYYCQQYYSTPRTFGQGTKVEIKRTVAAPSVFIFPPSDEQLKSGTASVVCLLNNFYPREAKVQWKVDNALQSGNSQESVTEQDSKDSTYSLSSTLTLSKADYEKHKVYACEVTHQGLSSPVTKSFNRGEC

SEQ ID NO: 13 - protein, 20 aa, Homo sapiens
MVLQTQVFISLLLWISGAYG

SEQ ID NO: 14 - protein, 518 aa, Artificial
  Heavy chain component of the recombinant fusion protein
QVQLQQWGAGLLKPSETLSLTCAVYGGSFSGYYWSWIRQPPGKGLEWIGEINHSGSTNYNPSLKSRVTISVETSKNQFSLKLSSVTAADTAVYYCARDKWTWYFDLWGRGTLVTVSSASTKGPSVFPLAPSSKSTSGGTAALGCLVKDYFPEPVTVSWNSGALTSGVHTFPAVLQSSGLYSLSSVVTVPSSSLGTQTYICNVNHKPSNTKVDKRVEPKSCDKTHTCPPCPAPEFLGGPAVFLFPPKPKDTLMISRTPEVTCVVVDVSHEDPEVKFNWYVDGVEVHNAKTKPREEQYNSTYRVVSVLTVLHQDWLNGKEYKCKVSNKALPAPIEKTISKAKGQPREPQVYTLPPSREEMTKNQVSLTCLVKGFYPSDIAVEWESNGQPENNYKTTPPVLDSDGSFFLYSKLTVDKSRWQQGNVFSCSVMHEALHAHYTQKSLSLSPGKGGGGSGGGGSSHLVKCAEKEKTFCVNGGECFMVKDLSNPSRYLCKCPNEFTGDRCQNYVMASFYKAEELYQ

SEQ ID NO: 15 - protein, 42 aa, Homo sapiens
HARKCNETAKSYCVNGGVCYYIEGINQLSCKCPNGFFGQRCL

SEQ ID NO: 16 - protein, 44 aa, Homo sapiens
HFKPCRDKDLAYCLNDGECFVIETLTGSHKHCRCKEGYQGVRCD

SEQ ID NO: 17 - protein, 42 aa, Homo sapiens
HEEPCGPSHKSFCLNGGLCYVIPTIPSPFCRCVENYTGARCE

SEQ ID NO: 18 - protein, 22 aa, Artificial Sequence
  EGF like domain consensus sequence
AEKEKTFCVNGECFMVKDLSNP